European Patent Application EP 4 324 913 A2, published February 21, 2024. Title: CULTURE MEDIA FOR STEM CELLS. Applicant: KONINKLIJKE NEDERLANDSE AKADEMIE VAN WETENSCHAPPEN. The sequence listing filed with the application follows.

SEQUENCE LISTING (30 sequences)

SEQ ID NO: 1 - protein, 17 aa, synthetic construct
  REGION 1..17: note = DSL peptide
CDDYYYGFGCNKFCRPR

SEQ ID NO: 2 - DNA, 22 bp, synthetic construct
  misc_feature 1..22: note = Primer
  source 1..22: mol_type = other DNA
gcagcattacctgctctacgtt

SEQ ID NO: 3 - DNA, 25 bp, synthetic construct
  misc_feature 1..25: note = Reverse primer
  source 1..25: mol_type = other DNA
gcttgataagctgatgctgtaattt

SEQ ID NO: 4 - skipped

SEQ ID NO: 5 - DNA, 18 bp, synthetic construct
  misc_feature 1..18: note = forward primer
  source 1..18: mol_type = other DNA
catggaccgcttcccata

SEQ ID NO: 6 - DNA, 19 bp, synthetic construct
  misc_feature 1..19: note = reverse primer
  source 1..19: mol_type = other DNA
ggcacctgtctgtccacat

SEQ ID NO: 7 - skipped

SEQ ID NO: 8 - DNA, 18 bp, synthetic construct
  misc_feature 1..18: note = Forward primer
  source 1..18: mol_type = other DNA
cagccaacgctgcttctc

SEQ ID NO: 9 - DNA, 18 bp, synthetic construct
  misc_feature 1..18: note = Reverse primer
  source 1..18: mol_type = other DNA
tggcatggaattgacagc

SEQ ID NO: 10 - skipped

SEQ ID NO: 11 - DNA, 21 bp, synthetic construct
  misc_feature 1..21: note = Forward primer
  source 1..21: mol_type = other DNA
ccgctactggtgtaatgatgg

SEQ ID NO: 12 - DNA, 22 bp, synthetic construct
  misc_feature 1..22: note = Reverse primer
  source 1..22: mol_type = other DNA
catcagcgatgttatcttgcag

SEQ ID NO: 13 - skipped

SEQ ID NO: 14 - DNA, 19 bp, synthetic construct
  misc_feature 1..19: note = Forward primer
  source 1..19: mol_type = other DNA
gccagctcatcaaggacag

SEQ ID NO: 15 - DNA, 21 bp, synthetic construct
  misc_feature 1..21: note = Reverse primer
  source 1..21: mol_type = other DNA
gcaggcatcgtagtagtgctg

SEQ ID NO: 16 - skipped

SEQ ID NO: 17 - DNA, 24 bp, synthetic construct
  misc_feature 1..24: note = Forward primer
  source 1..24: mol_type = other DNA
tgaccttgatttattttgcatacc

SEQ ID NO: 18 - DNA, 20 bp, synthetic construct
  misc_feature 1..20: note = Reverse primer
  source 1..20: mol_type = other DNA
cgagcaagacgttcagtcct

SEQ ID NO: 19 - DNA, 22 bp, synthetic construct
  misc_feature 1..22: note = Forward primer
  source 1..22: mol_type = other DNA
gcttgccacaacttcctaagat

SEQ ID NO: 20 - DNA, 22 bp, synthetic construct
  misc_feature 1..22: note = Reverse primer
  source 1..22: mol_type = other DNA
tcagtttagtcatggtggacga

SEQ ID NO: 21 - skipped

SEQ ID NO: 22 - DNA, 18 bp, synthetic construct
  misc_feature 1..18: note = Forward primer
  source 1..18: mol_type = other DNA
tgtggaaccgggaagatg

SEQ ID NO: 23 - DNA, 21 bp, synthetic construct
  misc_feature 1..21: note = Reverse primer
  source 1..21: mol_type = other DNA
gaccacaggtatggttctgga

SEQ ID NO: 24 - skipped

SEQ ID NO: 25 - DNA, 21 bp, synthetic construct
  misc_feature 1..21: note = Forward primer
  source 1..21: mol_type = other DNA
cgatccagaaagatgatggtc

SEQ ID NO: 26 - DNA, 19 bp, synthetic construct
  misc_feature 1..19: note = Reverse primer
  source 1..19: mol_type = other DNA
cggaagcctctgtctttcc

SEQ ID NO: 27 - skipped

SEQ ID NO: 28 - DNA, 19 bp, synthetic construct
  misc_feature 1..19: note = Forward primer
  source 1..19: mol_type = other DNA
tcctcctcagaccgctttt

SEQ ID NO: 29 - DNA, 21 bp, synthetic construct
  misc_feature 1..21: note = Reverse primer
  source 1..21: mol_type = other DNA
cctggttcatcatcgctaatc

SEQ ID NO: 30 - skipped